European Patent Application EP 4 223 785 A1, published August 9, 2023. Title: PHARMACEUTICAL COMPOSITION COMPRISING ANTIBODY-DRUG CONJUGATE, AND USE OF PHARMACEUTICAL COMPOSITION. Applicant: Jiangsu Hengrui Pharmaceuticals Co., Ltd. Shanghai Hengrui Pharmaceutical Co., Ltd. Application PCT/CN2021/122031. The sequence listing filed with the application follows.

SEQUENCE LISTING (55 sequences)

SEQ ID NO: 1 - protein, 261 aa, Homo sapiens
  Claudin18.2 protein
MAVTACQGLGFVVSLIGIAGIIAATCMDQWSTQDLYNNPVTAVFNYQGLWRSCVRESSGFTECRGYFTLLGLPAMLQAVRALMIVGIVLGAIGLLVSIFALKCIRIGSMEDSAKANMTLTSGIMFIVSGLCAIAGVSVFANMLVTNFWMSTANMYTGMGGMVQTVQTRYTFGAALFVGWVAGGLTLIGGVMMCIACRGLAPEETNYKAVSYHASGHSVAYKPGGFKASTGFGSNTKNKKIYDGGARTEDEVQSYPSKHDYV

SEQ ID NO: 2 - DNA, 3350 bp, Homo sapiens
  Claudin18.2
agaattgcgctgtccacttgtcgtgtggctctgtgtcgacactgtgcgccaccatggccgtgactgcctgtcagggcttggggttcgtggtttcactgattgggattgcgggcatcattgctgccacctgcatggaccagtggagcacccaagacttgtacaacaaccccgtaacagctgttttcaactaccaggggctgtggcgctcctgtgtccgagagagctctggcttcaccgagtgccggggctacttcaccctgctggggctgccagccatgctgcaggcagtgcgagccctgatgatcgtaggcatcgtcctgggtgccattggcctcctggtatccatctttgccctgaaatgcatccgcattggcagcatggaggactctgccaaagccaacatgacactgacctccgggatcatgttcattgtctcaggtctttgtgcaattgctggagtgtctgtgtttgccaacatgctggtgactaacttctggatgtccacagctaacatgtacaccggcatgggtgggatggtgcagactgttcagaccaggtacacatttggtgcggctctgttcgtgggctgggtcgctggaggcctcacactaattgggggtgtgatgatgtgcatcgcctgccggggcctggcaccagaagaaaccaactacaaagccgtttcttatcatgcctcaggccacagtgttgcctacaagcctggaggcttcaaggccagcactggctttgggtccaacaccaaaaacaagaagatatacgatggaggtgcccgcacagaggacgaggtacaatcttatccttccaagcacgactatgtgtaatgctctaagacctctcagcacgggcggaagaaactcccggagagctcacccaaaaaacaaggagatcccatctagatttcttcttgcttttgactcacagctggaagttagaaaagcctcgatttcatctttggagaggccaaatggtcttagcctcagtctctgtctctaaatattccaccataaaacagctgagttatttatgaattagaggctatagctcacattttcaatcctctatttctttttttaaatataactttctactctgatgagagaatgtggttttaatctctctctcacattttgatgatttagacagactccccctcttcctcctagtcaataaacccattgatgatctatttcccagcttatccccaagaaaacttttgaaaggaaagagtagacccaaagatgttattttctgctgtttgaattttgtctccccacccccaacttggctagtaataaacacttactgaagaagaagcaataagagaaagatatttgtaatctctccagcccatgatctcggttttcttacactgtgatcttaaaagttaccaaaccaaagtcattttcagtttgaggcaaccaaacctttctactgctgttgacatcttcttattacagcaacaccattctaggagtttcctgagctctccactggagtcctctttctgtcgcgggtcagaaattgtccctagatgaatgagaaaattattttttttaatttaagtcctaaatatagttaaaataaataatgttttagtaaaatgatacactatctctgtgaaatagcctcacccctacatgtggatagaaggaaatgaaaaaataattgctttgacattgtctatatggtactttgtaaagtcatgcttaagtacaaattccatgaaaagctcactgatcctaattctttccctttgaggtctctatggctctgattgtacatgatagtaagtgtaagccatgtaaaaagtaaataatgtctgggcacagtggctcacgcctgtaatcctagcactttgggaggctgaggaggaaggatcacttgagcccagaagttcgagactagcctgggcaacatggagaagccctgtctctacaaaatacagagagaaaaaatcagccagtcatggtggcctacacctgtagtcccagcattccgggaggctgaggtgggaggatcacttgagcccagggaggttggggctgcagtgagccatgatcacaccactgcactccagccaggtgacatagcgagatcctgtctaaaaaaataaaaaataaataatggaacacagcaagtcctaggaagtaggttaaaactaattctttaaaaaaaaaaaaaagttgagcctgaattaaatgtaatgtttccaagtgacaggtatccacatttgcatggttacaagccactgccagttagcagtagcactttcctggcactgtggtcggttttgttttgttttgctttgtttagagacggggtctcactttccaggctggcctcaaactcctgcactcaagcaattcttctaccctggcctcccaagtagctggaattacaggtgtgcgccatcacaactagctggtggtcagttttgttactctgagagctgttcacttctctgaattcacctagagtggttggaccatcagatgtttgggcaaaactgaaagctctttgcaaccacacaccttccctgagcttacatcactgcccttttgagcagaaagtctaaattccttccaagacagtagaattccatcccagtaccaaagccagataggccccctaggaaactgaggtaagagcagtctctaaaaactacccacagcagcattggtgcaggggaacttggccattaggttattatttgagaggaaagtcctcacatcaatagtacatatgaaagtgacctccaaggggattggtgaatactcataaggatcttcaggctgaacagactatgtctggggaaagaacggattatgccccattaaataacaagttgtgttcaagagtcagagcagtgagctcagaggcccttctcactgagacagcaacatttaaaccaaaccagaggaagtatttgtggaactcactgcctcagtttgggtaaaggatgagcagacaagtcaactaaagaaaaaagaaaagcaaggaggagggttgagcaatctagagcatggagtttgttaagtgctctctggatttgagttgaagagcatccatttgagttgaaggccacagggcacaatgagctctcccttctaccaccagaaagtccctggtcaggtctcaggtagtgcggtgtggctcagctgggtttttaattagcgcattctctatccaacatttaattgtttgaaagcctccatatagttagattgtgctttgtaattttgttgttgttgctctatcttattgtatatgcattgagtattaacctgaatgttttgttacttaaatattaaaaacactgttatcctacagtt

SEQ ID NO: 3 - protein, 120 aa, Mus musculus
  Heavy chain variable region of mAb1901 murine antibody
EVQLMESGGGLVKPGGSLKLSCAASGFTFSDYGIHWVRQAPEMGLEWIAYISRGSSTIYYADTVKGRFTMSRDNAKNTLFLQMTSLRSEDTAMYYCARGGYDTRNAMDYWGQGTSVTVSS

SEQ ID NO: 4 - protein, 113 aa, Mus musculus
  Light chain variable region of mAb1901 murine antibody
DIVMTQSPSSLSVSAGEKVTMSCKSSQSLLNSGNQKNYLAWYQQKPGQPPKLLIYGASTRASGVPDRFTGSGSGTDFTLTISSVQAEDLAIYHCQNDLYYPLTFGAGTKLELK

SEQ ID NO: 5 - protein, 118 aa, Mus musculus
  Heavy chain variable region of mAb1902 murine antibody
EVQLQESGAELVKPGASVKLSCKASGYIFTSYWMHWVKQRPGQGLEWIGMIHPNSGSTNYNEKFKGKATLTLDKSSSTAYMQLSSLPSEDSAVYYCARLKTGNSFDYWGQGTTLTVSS

SEQ ID NO: 6 - protein, 113 aa, Mus musculus
  Light chain variable region of mAb1902 murine antibody
DIVLTQSPSSLTVTAGEKVTMSCKSSQSLLNSGNQKNYLTWYQQKPGQPPKLLIYWASTRESGVPDRFTGSGSGTDFTLTISSVQAEDLAIYYCQNAYTYPFTFGSGTKLEIK

SEQ ID NO: 7 - protein, 330 aa, Homo sapiens [sequence omitted]

SEQ ID NO: 8 - protein, 107 aa, Homo sapiens [sequence omitted]

SEQ ID NO: 9 - protein, 5 aa, Artificial Sequence
  mAb1901 HCDR1
DYGIH

SEQ ID NO: 10 - protein, 17 aa, Artificial Sequence
  mAb1901 HCDR2
YISRGSSTIYYADTVKG

SEQ ID NO: 11 - protein, 11 aa, Artificial Sequence
  mAb1901 HCDR3
GGYDTRNAMDY

SEQ ID NO: 12 - protein, 17 aa, Artificial Sequence
  mAb1901 LCDR1
KSSQSLLNSGNQKNYLA

SEQ ID NO: 13 - protein, 7 aa, Artificial Sequence
  mAb1901 LCDR2
GASTRAS

SEQ ID NO: 14 - protein, 9 aa, Artificial Sequence
  mAb1901 LCDR3
QNDLYYPLT

SEQ ID NO: 15 - protein, 5 aa, Artificial Sequence
  mAb1902 HCDR1
SYWMH

SEQ ID NO: 16 - protein, 18 aa, Artificial Sequence
  mAb1902 HCDR2
MIHPNSGSTNYNEKFKGR

SEQ ID NO: 17 - protein, 9 aa, Artificial Sequence
  mAb1902 HCDR3
LKTGNSFDY

SEQ ID NO: 18 - protein, 17 aa, Artificial Sequence
  mAb1902 LCDR1
KSSQSLLNSGNQKNYLT

SEQ ID NO: 19 - protein, 7 aa, Artificial Sequence
  mAb1902 LCDR2
WASTRES

SEQ ID NO: 20 - protein, 9 aa, Artificial Sequence
  mAb1902 LCDR3
QNAYTYPFT

SEQ ID NO: 21 - protein, 113 aa, Artificial Sequence
  VL1
DIVMTQSPDSLAVSLGERATINCKSSQSLLNSGNQKNYLAWYQQKPGQPPKLLIYGASTRASGVPDRFSGSGSGTDFTLTISSLQAEDVAVYYCQNDLYYPLTFGQGTKLEIK

SEQ ID NO: 22 - protein, 113 aa, Artificial Sequence
  VL2
DIVMTQSPDSLAVSLGERATISCKSSQSLLNSGNQKNYLAWYQQKPGQPPKLLIYGASTRASGVPDRFSGSGSGTDFTLTISSLQAEDVAVYYCQNDLYYPLTFGQGTKLEIK

SEQ ID NO: 23 - protein, 113 aa, Artificial Sequence
  VL3
DIVMTQSPDSLAVSLGERATISCKSSQSLLNSGNQKNYLAWYQQKPGQPPKLLIYGASTRASGVPDRFSGSGSGTDFTLTISSLQAEDVAIYHCQNDLYYPLTFGQGTKLEIK

SEQ ID NO: 24 - protein, 120 aa, Artificial Sequence
  VH1
EVQLVESGGGLVQPGGSLRLSCAASGFTFSDYGIHWVRQAPGKGLEWVAYISRGSSTIYYADTVKGRFTISRDNAKNSLYLQMNSLRAEDTAVYYCARGGYDTRNAMDYWGQGTTVTVSS

SEQ ID NO: 25 - protein, 120 aa, Artificial Sequence
  VH2
EVQLVESGGGLVQPGGSLRLSCAASGFTFSDYGIHWVRQAPGKGLEWVAYISRGSSTIYYADTVKGRFTISRDNAKNSLYLQMTSLRAEDTAVYYCARGGYDTRNAMDYWGQGTTVTVSS

SEQ ID NO: 26 - protein, 120 aa, Artificial Sequence
  VH3
EVQLVESGGGLVQPGGSLRLSCAASGFTFSDYGIHWVRQAPGKGLEWIAYISRGSSTIYYADTVKGRFTISRDNAKNSLYLQMTSLRAEDTAVYYCARGGYDTRNAMDYWGQGTTVTVSS

SEQ ID NO: 27 - protein, 120 aa, Artificial Sequence
  VH4
EVQLVESGGGLVQPGGSLRLSCAASGFTFSDYGIHWVRQAPGKGLEWVAYISRGSSTIYYADTVKGRFTMSRDNAKNSLYLQMTSLRAEDTAVYYCARGGYDTRNAMDYWGQGTTVTVSS

SEQ ID NO: 28 - protein, 113 aa, Artificial Sequence
  VL11
DIVMTQSPDSLAVSLGERATINCKSSQSLLNSGNQKNYLTWYQQKPGQPPKLLIYWASTRESGVPDRFSGSGSGTDFTLTISSLQAEDVAVYYCQNAYTYPFTFGQGTKLEIK

SEQ ID NO: 29 - protein, 113 aa, Artificial Sequence
  VL12
DIVLTQSPDSLAVSLGERATINCKSSQSLLNSGNQKNYLTWYQQKPGQPPKLLIYWASTRESGVPDRFSGSGSGTDFTLTISSLQAEDVAVYYCQNAYTYPFTFGQGTKLEIK

SEQ ID NO: 30 - protein, 113 aa, Artificial Sequence
  VL13
DIVLTQSPDSLAVSLGERATISCKSSQSLLNSGNQKNYLTWYQQKPGQPPKLLIYWASTRESGVPDRFSGSGSGTDFTLTISSLQAEDVAVYYCQNAYTYPFTFGQGTKLEIK

SEQ ID NO: 31 - protein, 118 aa, Artificial Sequence
  VH11
EVQLVQSGAEVKKPGASVKVSCKASGYTFTSYWMHWVRQAPGQRLEWMGMIHPNSGSTNYNEKFKGRVTITRDTSASTAYMELSSLRSEDTAVYYCARLKTGNSFDYWGQGTTVTVSS

SEQ ID NO: 32 - protein, 118 aa, Artificial Sequence
  VH12
EVQLVQSGAEVKKPGASVKVSCKASGYTFTSYWMHWVRQAPGQRLEWMGMIHPNSGSTNYNEKFKGRVTLTLDKSASTAYMELSSLRSEDTAVYYCARLKTGNSFDYWGQGTTVTVSS

SEQ ID NO: 33 - protein, 118 aa, Artificial Sequence
  VH13
EVQLVQSGAEVKKPGASVKVSCKASGYTFTSYWMHWVRQAPGQRLEWIGMIHPNSGSTNYNEKFKGKATLTLDKSASTAYMELSSLRSEDTAVYYCARLKTGNSFDYWGQGTTVTVSS

SEQ ID NO: 34 - protein, 118 aa, Artificial Sequence
  VH14
EVQLVQSGAEVKKPGASVKVSCKASGYTFTSYWMHWVKQRPGQRLEWIGMIHPNSGSTNYNEKFKGKATLTLDKSASTAYMELSSLRSEDTAVYYCARLKTGNSFDYWGQGTTVTVSS

SEQ ID NO: 35 - protein, 450 aa, Artificial Sequence
  ch1901 heavy chain
EVQLMESGGGLVKPGGSLKLSCAASGFTFSDYGIHWVRQAPEMGLEWIAYISRGSSTIYYADTVKGRFTMSRDNAKNTLFLQMTSLRSEDTAMYYCARGGYDTRNAMDYWGQGTSVTVSSASTKGPSVFPLAPSSKSTSGGTAALGCLVKDYFPEPVTVSWNSGALTSGVHTFPAVLQSSGLYSLSSVVTVPSSSLGTQTYICNVNHKPSNTKVDKKVEPKSCDKTHTCPPCPAPELLGGPSVFLFPPKPKDTLMISRTPEVTCVVVDVSHEDPEVKFNWYVDGVEVHNAKTKPREEQYNSTYRVVSVLTVLHQDWLNGKEYKCKVSNKALPAPIEKTISKAKGQPREPQVYTLPPSRDELTKNQVSLTCLVKGFYPSDIAVEWESNGQPENNYKTTPPVLDSDGSFFLYSKLTVDKSRWQQGNVFSCSVMHEALHNHYTQKSLSLSPGK

SEQ ID NO: 36 - protein, 220 aa, Artificial Sequence
  ch1901 light chain
DIVMTQSPSSLSVSAGEKVTMSCKSSQSLLNSGNQKNYLAWYQQKPGQPPKLLIYGASTRASGVPDRFTGSGSGTDFTLTISSVQAEDLAIYHCQNDLYYPLTFGAGTKLELKRTVAAPSVFIFPPSDEQLKSGTASVVCLLNNFYPREAKVQWKVDNALQSGNSQESVTEQDSKDSTYSLSSTLTLSKADYEKHKVYACEVTHQGLSSPVTKSFNRGEC

SEQ ID NO: 37 - protein, 448 aa, Artificial Sequence
  ch1902 heavy chain
EVQLQESGAELVKPGASVKLSCKASGYIFTSYWMHWVKQRPGQGLEWIGMIHPNSGSTNYNEKFKGKATLTLDKSSSTAYMQLSSLPSEDSAVYYCARLKTGNSFDYWGQGTTLTVSSASTKGPSVFPLAPSSKSTSGGTAALGCLVKDYFPEPVTVSWNSGALTSGVHTFPAVLQSSGLYSLSSVVTVPSSSLGTQTYICNVNHKPSNTKVDKKVEPKSCDKTHTCPPCPAPELLGGPSVFLFPPKPKDTLMISRTPEVTCVVVDVSHEDPEVKFNWYVDGVEVHNAKTKPREEQYNSTYRVVSVLTVLHQDWLNGKEYKCKVSNKALPAPIEKTISKAKGQPREPQVYTLPPSRDELTKNQVSLTCLVKGFYPSDIAVEWESNGQPENNYKTTPPVLDSDGSFFLYSKLTVDKSRWQQGNVFSCSVMHEALHNHYTQKSLSLSPGK

SEQ ID NO: 38 - protein, 220 aa, Artificial Sequence
  ch1902 light chain
DIVLTQSPSSLTVTAGEKVTMSCKSSQSLLNSGNQKNYLTWYQQKPGQPPKLLIYWASTRESGVPDRFTGSGSGTDFTLTISSVQAEDLAIYYCQNAYTYPFTFGSGTKLEIKRTVAAPSVFIFPPSDEQLKSGTASVVCLLNNFYPREAKVQWKVDNALQSGNSQESVTEQDSKDSTYSLSSTLTLSKADYEKHKVYACEVTHQGLSSPVTKSFNRGEC

SEQ ID NO: 39 - protein, 220 aa, Artificial Sequence
  L1
DIVMTQSPDSLAVSLGERATINCKSSQSLLNSGNQKNYLAWYQQKPGQPPKLLIYGASTRASGVPDRFSGSGSGTDFTLTISSLQAEDVAVYYCQNDLYYPLTFGQGTKLEIKRTVAAPSVFIFPPSDEQLKSGTASVVCLLNNFYPREAKVQWKVDNALQSGNSQESVTEQDSKDSTYSLSSTLTLSKADYEKHKVYACEVTHQGLSSPVTKSFNRGEC

SEQ ID NO: 40 - protein, 220 aa, Artificial Sequence
  L2
DIVMTQSPDSLAVSLGERATISCKSSQSLLNSGNQKNYLAWYQQKPGQPPKLLIYGASTRASGVPDRFSGSGSGTDFTLTISSLQAEDVAVYYCQNDLYYPLTFGQGTKLEIKRTVAAPSVFIFPPSDEQLKSGTASVVCLLNNFYPREAKVQWKVDNALQSGNSQESVTEQDSKDSTYSLSSTLTLSKADYEKHKVYACEVTHQGLSSPVTKSFNRGEC

SEQ ID NO: 41 - protein, 220 aa, Artificial Sequence
  L3
DIVMTQSPDSLAVSLGERATISCKSSQSLLNSGNQKNYLAWYQQKPGQPPKLLIYGASTRASGVPDRFSGSGSGTDFTLTISSLQAEDVAIYHCQNDLYYPLTFGQGTKLEIKRTVAAPSVFIFPPSDEQLKSGTASVVCLLNNFYPREAKVQWKVDNALQSGNSQESVTEQDSKDSTYSLSSTLTLSKADYEKHKVYACEVTHQGLSSPVTKSFNRGEC

SEQ ID NO: 42 - protein, 450 aa, Artificial Sequence
  H1
EVQLVESGGGLVQPGGSLRLSCAASGFTFSDYGIHWVRQAPGKGLEWVAYISRGSSTIYYADTVKGRFTISRDNAKNSLYLQMNSLRAEDTAVYYCARGGYDTRNAMDYWGQGTTVTVSSASTKGPSVFPLAPSSKSTSGGTAALGCLVKDYFPEPVTVSWNSGALTSGVHTFPAVLQSSGLYSLSSVVTVPSSSLGTQTYICNVNHKPSNTKVDKKVEPKSCDKTHTCPPCPAPELLGGPSVFLFPPKPKDTLMISRTPEVTCVVVDVSHEDPEVKFNWYVDGVEVHNAKTKPREEQYNSTYRVVSVLTVLHQDWLNGKEYKCKVSNKALPAPIEKTISKAKGQPREPQVYTLPPSRDELTKNQVSLTCLVKGFYPSDIAVEWESNGQPENNYKTTPPVLDSDGSFFLYSKLTVDKSRWQQGNVFSCSVMHEALHNHYTQKSLSLSPGK

SEQ ID NO: 43 - protein, 450 aa, Artificial Sequence
  H2
EVQLVESGGGLVQPGGSLRLSCAASGFTFSDYGIHWVRQAPGKGLEWVAYISRGSSTIYYADTVKGRFTISRDNAKNSLYLQMTSLRAEDTAVYYCARGGYDTRNAMDYWGQGTTVTVSSASTKGPSVFPLAPSSKSTSGGTAALGCLVKDYFPEPVTVSWNSGALTSGVHTFPAVLQSSGLYSLSSVVTVPSSSLGTQTYICNVNHKPSNTKVDKKVEPKSCDKTHTCPPCPAPELLGGPSVFLFPPKPKDTLMISRTPEVTCVVVDVSHEDPEVKFNWYVDGVEVHNAKTKPREEQYNSTYRVVSVLTVLHQDWLNGKEYKCKVSNKALPAPIEKTISKAKGQPREPQVYTLPPSRDELTKNQVSLTCLVKGFYPSDIAVEWESNGQPENNYKTTPPVLDSDGSFFLYSKLTVDKSRWQQGNVFSCSVMHEALHNHYTQKSLSLSPGK

SEQ ID NO: 44 - protein, 450 aa, Artificial Sequence
  H3
EVQLVESGGGLVQPGGSLRLSCAASGFTFSDYGIHWVRQAPGKGLEWIAYISRGSSTIYYADTVKGRFTISRDNAKNSLYLQMTSLRAEDTAVYYCARGGYDTRNAMDYWGQGTTVTVSSASTKGPSVFPLAPSSKSTSGGTAALGCLVKDYFPEPVTVSWNSGALTSGVHTFPAVLQSSGLYSLSSVVTVPSSSLGTQTYICNVNHKPSNTKVDKKVEPKSCDKTHTCPPCPAPELLGGPSVFLFPPKPKDTLMISRTPEVTCVVVDVSHEDPEVKFNWYVDGVEVHNAKTKPREEQYNSTYRVVSVLTVLHQDWLNGKEYKCKVSNKALPAPIEKTISKAKGQPREPQVYTLPPSRDELTKNQVSLTCLVKGFYPSDIAVEWESNGQPENNYKTTPPVLDSDGSFFLYSKLTVDKSRWQQGNVFSCSVMHEALHNHYTQKSLSLSPGK

SEQ ID NO: 45 - protein, 450 aa, Artificial Sequence
  H4
EVQLVESGGGLVQPGGSLRLSCAASGFTFSDYGIHWVRQAPGKGLEWVAYISRGSSTIYYADTVKGRFTMSRDNAKNSLYLQMTSLRAEDTAVYYCARGGYDTRNAMDYWGQGTTVTVSSASTKGPSVFPLAPSSKSTSGGTAALGCLVKDYFPEPVTVSWNSGALTSGVHTFPAVLQSSGLYSLSSVVTVPSSSLGTQTYICNVNHKPSNTKVDKKVEPKSCDKTHTCPPCPAPELLGGPSVFLFPPKPKDTLMISRTPEVTCVVVDVSHEDPEVKFNWYVDGVEVHNAKTKPREEQYNSTYRVVSVLTVLHQDWLNGKEYKCKVSNKALPAPIEKTISKAKGQPREPQVYTLPPSRDELTKNQVSLTCLVKGFYPSDIAVEWESNGQPENNYKTTPPVLDSDGSFFLYSKLTVDKSRWQQGNVFSCSVMHEALHNHYTQKSLSLSPGK

SEQ ID NO: 46 - protein, 220 aa, Artificial Sequence
  L11
DIVMTQSPDSLAVSLGERATINCKSSQSLLNSGNQKNYLTWYQQKPGQPPKLLIYWASTRESGVPDRFSGSGSGTDFTLTISSLQAEDVAVYYCQNAYTYPFTFGQGTKLEIKRTVAAPSVFIFPPSDEQLKSGTASVVCLLNNFYPREAKVQWKVDNALQSGNSQESVTEQDSKDSTYSLSSTLTLSKADYEKHKVYACEVTHQGLSSPVTKSFNRGEC

SEQ ID NO: 47 - protein, 220 aa, Artificial Sequence
  L12
DIVLTQSPDSLAVSLGERATINCKSSQSLLNSGNQKNYLTWYQQKPGQPPKLLIYWASTRESGVPDRFSGSGSGTDFTLTISSLQAEDVAVYYCQNAYTYPFTFGQGTKLEIKRTVAAPSVFIFPPSDEQLKSGTASVVCLLNNFYPREAKVQWKVDNALQSGNSQESVTEQDSKDSTYSLSSTLTLSKADYEKHKVYACEVTHQGLSSPVTKSFNRGEC

SEQ ID NO: 48 - protein, 220 aa, Artificial Sequence
  L13
DIVLTQSPDSLAVSLGERATISCKSSQSLLNSGNQKNYLTWYQQKPGQPPKLLIYWASTRESGVPDRFSGSGSGTDFTLTISSLQAEDVAVYYCQNAYTYPFTFGQGTKLEIKRTVAAPSVFIFPPSDEQLKSGTASVVCLLNNFYPREAKVQWKVDNALQSGNSQESVTEQDSKDSTYSLSSTLTLSKADYEKHKVYACEVTHQGLSSPVTKSFNRGEC

SEQ ID NO: 49 - protein, 448 aa, Artificial Sequence
  H11
EVQLVQSGAEVKKPGASVKVSCKASGYTFTSYWMHWVRQAPGQRLEWMGMIHPNSGSTNYNEKFKGRVTITRDTSASTAYMELSSLRSEDTAVYYCARLKTGNSFDYWGQGTTVTVSSASTKGPSVFPLAPSSKSTSGGTAALGCLVKDYFPEPVTVSWNSGALTSGVHTFPAVLQSSGLYSLSSVVTVPSSSLGTQTYICNVNHKPSNTKVDKKVEPKSCDKTHTCPPCPAPELLGGPSVFLFPPKPKDTLMISRTPEVTCVVVDVSHEDPEVKFNWYVDGVEVHNAKTKPREEQYNSTYRVVSVLTVLHQDWLNGKEYKCKVSNKALPAPIEKTISKAKGQPREPQVYTLPPSRDELTKNQVSLTCLVKGFYPSDIAVEWESNGQPENNYKTTPPVLDSDGSFFLYSKLTVDKSRWQQGNVFSCSVMHEALHNHYTQKSLSLSPGK

SEQ ID NO: 50 - protein, 448 aa, Artificial Sequence
  H12
EVQLVQSGAEVKKPGASVKVSCKASGYTFTSYWMHWVRQAPGQRLEWMGMIHPNSGSTNYNEKFKGRVTLTLDKSASTAYMELSSLRSEDTAVYYCARLKTGNSFDYWGQGTTVTVSSASTKGPSVFPLAPSSKSTSGGTAALGCLVKDYFPEPVTVSWNSGALTSGVHTFPAVLQSSGLYSLSSVVTVPSSSLGTQTYICNVNHKPSNTKVDKKVEPKSCDKTHTCPPCPAPELLGGPSVFLFPPKPKDTLMISRTPEVTCVVVDVSHEDPEVKFNWYVDGVEVHNAKTKPREEQYNSTYRVVSVLTVLHQDWLNGKEYKCKVSNKALPAPIEKTISKAKGQPREPQVYTLPPSRDELTKNQVSLTCLVKGFYPSDIAVEWESNGQPENNYKTTPPVLDSDGSFFLYSKLTVDKSRWQQGNVFSCSVMHEALHNHYTQKSLSLSPGK

SEQ ID NO: 51 - protein, 448 aa, Artificial Sequence
  H13
EVQLVQSGAEVKKPGASVKVSCKASGYTFTSYWMHWVRQAPGQRLEWIGMIHPNSGSTNYNEKFKGKATLTLDKSASTAYMELSSLRSEDTAVYYCARLKTGNSFDYWGQGTTVTVSSASTKGPSVFPLAPSSKSTSGGTAALGCLVKDYFPEPVTVSWNSGALTSGVHTFPAVLQSSGLYSLSSVVTVPSSSLGTQTYICNVNHKPSNTKVDKKVEPKSCDKTHTCPPCPAPELLGGPSVFLFPPKPKDTLMISRTPEVTCVVVDVSHEDPEVKFNWYVDGVEVHNAKTKPREEQYNSTYRVVSVLTVLHQDWLNGKEYKCKVSNKALPAPIEKTISKAKGQPREPQVYTLPPSRDELTKNQVSLTCLVKGFYPSDIAVEWESNGQPENNYKTTPPVLDSDGSFFLYSKLTVDKSRWQQGNVFSCSVMHEALHNHYTQKSLSLSPGK

SEQ ID NO: 52 - protein, 448 aa, Artificial Sequence
  H14
EVQLVQSGAEVKKPGASVKVSCKASGYTFTSYWMHWVKQRPGQRLEWIGMIHPNSGSTNYNEKFKGKATLTLDKSASTAYMELSSLRSEDTAVYYCARLKTGNSFDYWGQGTTVTVSSASTKGPSVFPLAPSSKSTSGGTAALGCLVKDYFPEPVTVSWNSGALTSGVHTFPAVLQSSGLYSLSSVVTVPSSSLGTQTYICNVNHKPSNTKVDKKVEPKSCDKTHTCPPCPAPELLGGPSVFLFPPKPKDTLMISRTPEVTCVVVDVSHEDPEVKFNWYVDGVEVHNAKTKPREEQYNSTYRVVSVLTVLHQDWLNGKEYKCKVSNKALPAPIEKTISKAKGQPREPQVYTLPPSRDELTKNQVSLTCLVKGFYPSDIAVEWESNGQPENNYKTTPPVLDSDGSFFLYSKLTVDKSRWQQGNVFSCSVMHEALHNHYTQKSLSLSPGK

SEQ ID NO: 53 - protein, 448 aa, Artificial Sequence
  IMAB-362 heavy chain
QVQLQQPGAELVRPGASVKLSCKASGYTFTSYWINWVKQRPGQGLEWIGNIYPSDSYTNYNQKFKDKATLTVDKSSSTAYMQLSSPTSEDSAVYYCTRSWRGNSFDYWGQGTTLTVSSASTKGPSVFPLAPSSKSTSGGTAALGCLVKDYFPEPVTVSWNSGALTSGVHTFPAVLQSSGLYSLSSVVTVPSSSLGTQTYICNVNHKPSNTKVDKRVEPKSCDKTHTCPPCPAPELLGGPSVFLFPPKPKDTLMISRTPEVTCVVVDVSHEDPEVKFNWYVDGVEVHNAKTKPREEQYNSTYRVVSVLTVLHQDWLNGKEYKCKVSNKALPAPIEKTISKAKGQPREPQVYTLPPSREEMTKNQVSLTCLVKGFYPSDIAVEWESNGQPENNYKTTPPVLDSDGSFFLYSKLTVDKSRWQQGNVFSCSVMHEALHNHYTQKSLSLSPGK

SEQ ID NO: 54 - protein, 220 aa, Artificial Sequence
  IMAB-362 light chain
DIVMTQSPSSLTVTAGEKVTMSCKSSQSLLNSGNQKNYLTWYQQKPGQPPKLLIYWASTRESGVPDRFTGSGSGTDFTLTISSVQAEDLAVYYCQNDYSYPFTFGSGTKLEIKRTVAAPSVFIFPPSDEQLKSGTASVVCLLNNFYPREAKVQWKVDNALQSGNSQESVTEQDSKDSTYSLSSTLTLSKADYEKHKVYACEVTHQGLSSPVTKSFNRGEC

SEQ ID NO: 55 - protein, 4 aa, Artificial Sequence
  Tetrapeptide linker
GGFG